European Patent Specification EP 3 743 094 B1, published March 27, 2024. Title: MDA-7 Secretory Variants and Methods of Use. Applicant: Virginia Commonwealth University Fisher, Paul B. Menezes, Mitchell E. Bhoopathy, Praveen Das, Swadesh Emdad, Luni Sarkar, Devanand Pradhan, Anjan K. Wang, Xiang-Yang. The sequence listing filed with the application follows.

SEQUENCE LISTING (20 sequences)

SEQ ID NO: 1 - DNA, 621 bp, Artificial sequence
  Synthetic polynucleotide
atgaattttcaacagaggctgcaaagcctgtggactttagccagacccttctgccctcctttgctggcgacagcctctcaaatgcagatggttgtgctcccttgcctgggttttaccctgcttctctggagccaggtatcaggggcccagggccaagaattccactttgggccctgccaagtgaagggggttgttccccagaaactgtgggaagccttctgggctgtgaaagacactatgcaagctcaggataacatcacgagtgcccggctgctgcagcaggaggttctgcagaacgtctcggatgctgagagctgttaccttgtccacaccctgctggagttctacttgaaaactgttttcaaaaactaccacaatagaacagttgaagtcaggactctgaagtcattctctactctggccaacaactttgttctcatcgtgtcacaactgcaacccagtcaagaaaatgagatgttttccatcagagacagtgcacacaggcggttcctgctattccggagagcatttaaacagttggacgtagaagcagctctgaccaaagcccttggggaagtggacattcttctgacctggatgcagaaattctacaagctctga

SEQ ID NO: 2 - protein, 206 aa, Artificial sequence
  Synthetic polypeptide
MNFQQRLQSLWTLARPFCPPLLATASQMQMVVLPCLGFTLLLWSQVSGAQGQEFHFGPCQVKGVVPQKLWEAFWAVKDTMQAQDNITSARLLQQEVLQNVSDAESCYLVHTLLEFYLKTVFKNYHNRTVEVRTLKSFSTLANNFVLIVSQLQPSQENEMFSIRDSAHRRFLLFRRAFKQLDVEAALTKALGEVDILLTWMQKFYKL

SEQ ID NO: 3 - protein, 157 aa, Artificial sequence
  Synthetic polypeptide
QGQEFHFGPCQVKGVVPQKLWEAFWAVKDTMQAQDNITSARLLQQEVLQNVSDAESCYLVHTLLEFYLKTVFKNYHNRTVEVRTLKSFSTLANNFVLIVSQLQPSQENEMFSIRDSAHRRFLLFRRAFKQLDVEAALTKALGEVDILLTWMQKFYKL

SEQ ID NO: 4 - protein, 103 aa, Artificial sequence
  Synthetic polypeptide
ESCYLVHTLLEFYLKTVFKNYHNRTVEVRTLKSFSTLANNFVLIVSQLQPSQENEMFSIRDSAHRRFLLFRRAFKQLDVEAALTKALGEVDILLTWMQKFYKL

SEQ ID NO: 5 - protein, 24 aa, Artificial sequence
  Synthetic polypeptide
MALWMRLLPLLALLALWGPDPAAA

SEQ ID NO: 6 - DNA, 582 bp, Artificial sequence
  Synthetic polynucleotide
atggcgctgtggatgcgcctgctgccgctgctggcgctgctggcgctgtggggcccagatccggcggcggcgcatcaccatcaccatcacgagaacctgtacttccagggcatgcaagaattccactttgggccctgccaagtgaagggggttgttccccagaaactgtgggaagccttctgggctgtgaaagacactatgcaagctcaggataacatcacgagtgcccggctgctgcagcaggaggttctgcagaacgtctcggatgctgagagctgttaccttgtccacaccctgctggagttctacttgaaaactgttttcaaaaactaccacaatagaacagttgaagtcaggactctgaagtcattctctactctggccaacaactttgttctcatcgtgtcacaactgcaacccagtcaagaaaatgagatgttttccatcagagacagtgcacacaggcggttcctgctattccggagagcattcaaacagttggacgtagaagcagctctgaccaaagcccttggggaagtggacattcttctgacctggatgcagaaattctacaagctctag

SEQ ID NO: 7 - DNA, 567 bp, Artificial sequence
  Synthetic polynucleotide
atgacagtgctggcgccagcctggagcccaacaacctatctcctcctgctgctgctgctgagcggatccatgcaagaattccactttgggccctgccaagtgaagggggttgttccccagaaactgtgggaagccttctgggctgtgaaagacactatgcaagctcaggataacatcacgagtgcccggctgctgcagcaggaggttctgcagaacgtctcggatgctgagagctgttaccttgtccacaccctgctggagttctacttgaaaactgttttcaaaaactaccacaatagaacagttgaagtcaggactctgaagtcattctctactctggccaacaactttgttctcatcgtgtcacaactgcaacccagtcaagaaaatgagatgttttccatcagagacagtgcacacaggcggtttctgctattccggagagcattcaaacagttggacgtagaagcagctctgaccaaagcccttggggaagtggacattcttctgacctggatgcagaaattctacaagctcgggggttctcatcatcatcatcatcattga

SEQ ID NO: 8 - DNA, 561 bp, Artificial sequence
  Synthetic polynucleotide
atgagagcctggatcttttttctgctctgcctcgctggcagagccctggctcatcaccatcaccatcacgagaacctgtacttccagggcatgcaagaattccactttgggccctgccaagtgaagggggttgttccccagaaactgtgggaagccttctgggctgtgaaagacactatgcaagctcaggataacatcacgagtgcccggctgctgcagcaggaggttctgcagaacgtctcggatgctgagagctgttaccttgtccacaccctgctggagttctacttgaaaactgttttcaaaaactaccacaatagaacagttgaagtcaggactctgaagtcattctctactctggccaacaactttgttctcatcgtgtcacaactgcaacccagtcaagaaaatgagatgttttccatcagagacagtgcacacaggcggtttctgctattccggagagcattcaaacagttggacgtagaagcagctctgaccaaagcccttggggaagtggacattcttctgacctggatgcagaaattctacaagctctga

SEQ ID NO: 9 - DNA, 513 bp, Artificial sequence
  Synthetic polynucleotide
atgcagctgctgtcatgcatcgcattgatcttggcgctggtgatgcaagaattccactttgggccctgccaagtgaagggggttgttccccagaaactgtgggaagccttctgggctgtgaaagacactatgcaagctcaggataacatcacgagtgcccggctgctgcagcaggaggttctgcagaacgtctcggatgctgagagctgttaccttgtccacaccctgctggagttctacttgaaaactgttttcaaaaactaccacaatagaacagttgaagtcaggactctgaagtcattctctactctggccaacaactttgttctcatcgtgtcacaactgcaacccagtcaagaaaatgagatgttttccatcagagacagtgcacacaggcggtttctgctattccggagagcattcaaacagttggacgtagaagcagctctgaccaaagcccttggggaagtggacattcttctgacctggatgcagaaattctacaagctctga

SEQ ID NO: 10 - DNA, 621 bp, Artificial sequence
  Synthetic polynucleotide
atgaattttcaacagaggctgcaaagcctgtggactttagccagacccttctgccctcctttgctggcgacagcctctcaaatgcagatggttgtgctcccttgcctgggttttaccctgcttctctggagccaggtatcaggggcccagggccaagaattccactttgggccctgccaagtgaagggggttgttccccagaaactgtgggaagccttctgggctgtgaaagacactatgcaagctcaggataacatcacgagtgcccggctgctgcagcaggaggttctgcagaacgtctcggatgctgagagctgttaccttgtccacaccctgctggagttctacttgaaaactgttttcagaaactaccacaatagaacagttgaagtcaggactctgaagtcattctctactctggccaacaactttgttctcatcgtgtcacaactgcaacccagtcaagaaaatgagatgttttccatcagagacagtgcacacaggcggtttctgctattccggagagcattcaaacagttggacgtagaagcagctctgaccaaagcccttggggaagtggacattcttctgacctggatgcagaaattctacaagctctga

SEQ ID NO: 11 - DNA, 582 bp, Artificial sequence
  Synthetic polynucleotide
atggcgctgtggatgcgcctgctgccgctgctggcgctgctggcgctgtggggcccagatccggcggcggcgcatcaccatcaccatcacgagaacctgtacttccagggcatgcaagaattccactttgggccctgccaagtgaagggggttgttccccagaaactgtgggaagccttctgggctgtgaaagacactatgcaagctcaggataacatcacgagtgcccggctgctgcagcaggaggttctgcagaacgtctcggatgctgagagctgttaccttgtccacaccctgctggagttctacttgaaaactgttttcagaaactaccacaatagaacagttgaagtcaggactctgaagtcattctctactctggccaacaactttgttctcatcgtgtcacaactgcaacccagtcaagaaaatgagatgttttccatcagagacagtgcacacaggcggttcctgctattccggagagcattcaaacagttggacgtagaagcagctctgaccaaagcccttggggaagtggacattcttctgacctggatgcagaaattctacaagctctag

SEQ ID NO: 12 - DNA, 426 bp, Artificial sequence
  Synthetic polynucleotide
atggcgctgtggatgcgcctgctgccgctgctggcgctgctggcgctgtggggcccagatccggcggcggcgcatcaccatcaccatcacgagaacctgtacttccagggcatggagagctgttaccttgtccacaccctgctggagttctacttgaaaactgttttcaaaaactaccacaatagaacagttgaagtcaggactctgaagtcattctctactctggccaacaactttgttctcatcgtgtcacaactgcaacccagtcaagaaaatgagatgttttccatcagagacagtgcacacaggcggttcctgctattccggagagcattcaaacagttggacgtagaagcagctctgaccaaagcccttggggaagtggacattcttctgacctggatgcagaaattctacaagctctag

SEQ ID NO: 13 - DNA, 357 bp, Artificial sequence
  Synthetic polynucleotide
atgcagctgctgtcatgcatcgcattgatcttggcgctggtgatggagagctgttaccttgtccacaccctgctggagttctacttgaaaactgttttcaaaaactaccacaatagaacagttgaagtcaggactctgaagtcattctctactctggccaacaactttgttctcatcgtgtcacaactgcaacccagtcaagaaaatgagatgttttccatcagagacagtgcacacaggcggtttctgctattccggagagcattcaaacagttggacgtagaagcagctctgaccaaagcccttggggaagtggacattcttctgacctggatgcagaaattctacaagctctga

SEQ ID NO: 14 - DNA, 408 bp, Artificial sequence
  Synthetic polynucleotide
atgacagtgctggcgccagcctggagcccaacaacctatctcctcctgctgctgctgctgagcggatccgagagctgttaccttgtccacaccctgctggagttctacttgaaaactgttttcaaaaactaccacaatagaacagttgaagtcaggactctgaagtcattctctactctggccaacaactttgttctcatcgtgtcacaactgcaacccagtcaagaaaatgagatgttttccatcagagacagtgcacacaggcggtttctgctattccggagagcattcaaacagttggacgtagaagcagctctgaccaaagcccttggggaagtggacattcttctgacctggatgcagaaattctacaagctcgggggttctcatcatcatcatcatcattga

SEQ ID NO: 15 - DNA, 471 bp, Artificial sequence
  Synthetic polynucleotide
atgaattttcaacagaggctgcaaagcctgtggactttagccagacccttctgccctcctttgctggcgacagcctctcaaatgcagatggttgtgctcccttgcctgggttttaccctgcttctctggagccaggtatcaggggcccagggcggatccgagagctgttaccttgtccacaccctgctggagttctacttgaaaactgttttcaaaaactaccacaatagaacagttgaagtcaggactctgaagtcattctctactctggccaacaactttgttctcatcgtgtcacaactgcaacccagtcaagaaaatgagatgttttccatcagagacagtgcacacaggcggtttctgctattccggagagcattcaaacagttggacgtagaagcagctctgaccaaagcccttggggaagtggacattcttctgacctggatgcagaaattctacaagctctga

SEQ ID NO: 16 - DNA, 408 bp, Artificial sequence
  Synthetic polynucleotide
atgacagtgctggcgccagcctggagcccaacaacctatctcctcctgctgctgctgctgagcggatccgagagctgttaccttgtccacaccctgctggagttctacttgaaaactgttttcagaaactaccacaatagaacagttgaagtcaggactctgaagtcattctctactctggccaacaactttgttctcatcgtgtcacaactgcaacccagtcaagaaaatgagatgttttccatcagagacagtgcacacaggcggtttctgctattccggagagcattcaaacagttggacgtagaagcagctctgaccaaagcccttggggaagtggacattcttctgacctggatgcagaaattctacaagctcgggggttctcatcatcatcatcatcattga

SEQ ID NO: 17 - DNA, 426 bp, Artificial sequence
  Synthetic polynucleotide
atggcgctgtggatgcgcctgctgccgctgctggcgctgctggcgctgtggggcccagatccggcggcggcgcatcaccatcaccatcacgagaacctgtacttccagggcatggagagctgttaccttgtccacaccctgctggagttctacttgaaaactgttttcagaaactaccacaatagaacagttgaagtcaggactctgaagtcattctctactctggccaacaactttgttctcatcgtgtcacaactgcaacccagtcaagaaaatgagatgttttccatcagagacagtgcacacaggcggttcctgctattccggagagcattcaaacagttggacgtagaagcagctctgaccaaagcccttggggaagtggacattcttctgacctggatgcagaaattctacaagctctag

SEQ ID NO: 18 - protein, 103 aa, Artificial sequence
  Synthetic polypeptide
ESCYLVHTLLEFYLKTVFRNYHNRTVEVRTLKSFSTLANNFVLIVSQLQPSQENEMFSIRDSAHRRFLLFRRAFKQLDVEAALTKALGEVDILLTWMQKFYKL

SEQ ID NO: 19 - DNA, 47 bp, Artificial sequence
  Synthetic polynucleotide
caactgttctattgtggtagtttctgaaaacagttttcaagtagaac

SEQ ID NO: 20 - DNA, 47 bp, Artificial sequence
  Synthetic polynucleotide
gttctacttgaaaactgttttcagaaactaccacaatagaacagttg